European Patent Application EP 4 166 566 A1, published April 19, 2023. Title: CHIMERIC ANTIGEN RECEPTOR AND USE THEREOF. Applicant: Center for Excellence in Molecular Cell Science, Chinese Academy of Sciences. The sequence listing filed with the application follows.

SEQUENCE LISTING (10 sequences)

SEQ ID NO: 1 - protein, 55 aa, Artificial Sequence
KNRKAKAKPVTRGAGAGGRQRGQNKERPPPVPNPDYEPIRKGQRDLYSGLNQRRI

SEQ ID NO: 2 - protein, 41 aa, Artificial Sequence
RSKRSRLLHSDYMNMTPRRPGPTRKHYQPYAPPRDFAAYRS

SEQ ID NO: 3 - protein, 112 aa, Artificial Sequence
RVKFSRSADAPAYQQGQNQLYNELNLGRREEYDVLDKRRGRDPEMGGKPRRKNPQEGLYNELQKDKMAEAYSEIGMKGERRRGKGHDGLYQGLSTATKDTYDALHMQALPPR

SEQ ID NO: 4 - protein, 27 aa, Artificial Sequence
FWVLVVVGGVLACYSLLVTVAFIIFWV

SEQ ID NO: 5 - protein, 813 aa, Artificial Sequence
MVSKGEELFTGVVPILVELDGDVNGHKFSVSGEGEGDATYGKLTLKFICTTGKLPVPWPTLVTTLTYGVQCFSRYPDHMKQHDFFKSAMPEGYVQERTIFFKDDGNYKTRAEVKFEGDTLVNRIELKGIDFKEDGNILGHKLEYNYNSHNVYIMADKQKNGIKVNFKIRHNIEDGSVQLADHYQQNTPIGDGPVLLPDNHYLSTQSALSKDPNEKRDHMVLLEFVTAAGITLGMDELYKGSGEGRGSLLTCGDVEENPGPMLLLVTSLLLCELPHPAFLLIPYPYDVPDYADIQMTQTTSSLSASLGDRVTISCRASQDISKYLNWYQQKPDGTVKLLIYHTSRLHSGVPSRFSGSGSGTDYSLTISNLEQEDIATYFCQQGNTLPYTFGGGTKLEITGSTSGSGKPGSGEGSTKGEVKLQESGPGLVAPSQSLSVTCTVSGVSLPDYGVSWIRQPPRKGLEWLGVIWGSETTYYNSALKSRLTIIKDNSKSQVFLKMNSLQTDDTAIYYCAKHYYYGGSYAMDYWGQGTSVTVSSAAAIEVMYPPPYLDNEKSNGTIIHVKGKHLCPSPLFPGPSKPFWVLVVVGGVLACYSLLVTVAFIIFWVKNRKAKAKPVTRGAGAGGRQRGQNKERPPPVPNPDYEPIRKGQRDLYSGLNQRRIRSKRSRLLHSDYMNMTPRRPGPTRKHYQPYAPPRDFAAYRSRVKFSRSADAPAYQQGQNQLYNELNLGRREEYDVLDKRRGRDPEMGGKPRRKNPQEGLYNELQKDKMAEAYSEIGMKGERRRGKGHDGLYQGLSTATKDTYDALHMQALPPR

SEQ ID NO: 6 - protein, 808 aa, Artificial Sequence
MVSKGEELFTGVVPILVELDGDVNGHKFSVSGEGEGDATYGKLTLKFICTTGKLPVPWPTLVTTLTYGVQCFSRYPDHMKQHDFFKSAMPEGYVQERTIFFKDDGNYKTRAEVKFEGDTLVNRIELKGIDFKEDGNILGHKLEYNYNSHNVYIMADKQKNGIKVNFKIRHNIEDGSVQLADHYQQNTPIGDGPVLLPDNHYLSTQSALSKDPNEKRDHMVLLEFVTAAGITLGMDELYKGSGEGRGSLLTCGDVEENPGPMLLLVTSLLLCELPHPAFLLIPYPYDVPDYAQVQLQQSGPELEKPGASVKISCKASGYSFTGYTMNWVKQSHGKSLEWIGLITPYNGASSYNQKFRGKATLTVDKSSSTAYMDLLSLTSEDSAVYFCARGGYDGRGFDYWGQGTTVTVSSGGGGSGGGGSSGGGSDIELTQSPAIMSASPGEKVTMTCSASSSVSYMHWYQQKSGTSPKRWIYDTSKLASGVPGRFSGSGSGNSYSLTISSVEAEDDATYYCQQWSKHPLTYGAGTKLEIKAAAIEVMYPPPYLDNEKSNGTIIHVKGKHLCPSPLFPGPSKPFWVLVVVGGVLACYSLLVTVAFIIFWVKNRKAKAKPVTRGAGAGGRQRGQNKERPPPVPNPDYEPIRKGQRDLYSGLNQRRIRSKRSRLLHSDYMNMTPRRPGPTRKHYQPYAPPRDFAAYRSRVKFSRSADAPAYQQGQNQLYNELNLGRREEYDVLDKRRGRDPEMGGKPRRKNPQEGLYNELQKDKMAEAYSEIGMKGERRRGKGHDGLYQGLSTATKDTYDALHMQALPPR

SEQ ID NO: 7 - DNA, 2442 bp, Artificial Sequence
atggtgagcaagggcgaggagctgttcaccggggtggtgcccatcctggtcgagctggacggcgacgtaaacggccacaagttcagcgtgtccggcgagggcgagggcgatgccacctacggcaagctgaccctgaagttcatctgcaccaccggcaagctgcccgtgccctggcccaccctcgtgaccaccctgacctacggcgtgcagtgcttcagccgctaccccgaccacatgaagcagcacgacttcttcaagtccgccatgcccgaaggctacgtccaggagcgcaccatcttcttcaaggacgacggcaactacaagacccgcgccgaggtgaagttcgagggcgacaccctggtgaaccgcatcgagctgaagggcatcgacttcaaggaggacggcaacatcctggggcacaagctggagtacaactacaacagccacaacgtctatatcatggccgacaagcagaagaacggcatcaaggtgaacttcaagatccgccacaacatcgaggacggcagcgtgcagctcgccgaccactaccagcagaacacccccatcggcgacggccccgtgctgctgcccgacaaccactacctgagcacccagtccgccctgagcaaagaccccaacgagaagcgcgatcacatggtcctgctggagttcgtgaccgccgccgggatcactctcggcatggacgagctgtacaagggaagcggagagggcagaggaagtctgctaacatgcggtgacgtcgaggagaatcctggacctatgcttctcctggtgacaagccttctgctctgtgagttaccacacccagcattcctcctgatcccatacccctacgacgtgcccgactacgccgacatccagatgacacagactacatcctccctgtctgcctctctgggagacagagtcaccatcagttgcagggcaagtcaggacattagtaaatatttaaattggtatcagcagaaaccagatggaactgttaaactcctgatctaccatacatcaagattacactcaggagtcccatcaaggttcagtggcagtgggtctggaacagattattctctcaccattagcaacctggagcaagaagatattgccacttacttttgccaacagggtaatacgcttccgtacacgttcggaggggggactaagttggaaataacaggctccacctctggatccggcaagcccggatctggcgagggatccaccaagggcgaggtgaaactgcaggagtcaggacctggcctggtggcgccctcacagagcctgtccgtcacatgcactgtctcaggggtctcattacccgactatggtgtaagctggattcgccagcctccacgaaagggtctggagtggctgggagtaatatggggtagtgaaaccacatactataattcagctctcaaatccagactgaccatcatcaaggacaactccaagagccaagttttcttaaaaatgaacagtctgcaaactgatgacacagccatttactactgtgccaaacattattactacggtggtagctatgctatggactactggggtcaaggaacctcagtcaccgtctcctcagcggccgcaattgaagttatgtatcctcctccttacctagacaatgagaagagcaatggaaccattatccatgtgaaagggaaacacctttgtccaagtcccctatttcccggaccttctaagcccttttgggtgctggtggtggttgggggagtcctggcttgctatagcttgctagtaacagtggcctttattattttctgggtgaagaatagaaaggccaaggccaagcctgtgacacgaggagcgggtgctggcggcaggcaaaggggacaaaacaaggagaggccaccacctgttcccaacccagactatgagcccatccggaaaggccagcgggacctgtattctggcctgaatcagagacgcatcaggagtaagaggagcaggctcctgcacagtgactacatgaacatgactccccgccgccccgggcccacccgcaagcattaccagccctatgccccaccacgcgacttcgcagcctatcgctccagagtgaagttcagcaggagcgcagacgcccccgcgtaccagcagggccagaaccagctctataacgagctcaatctaggacgaagagaggagtacgatgttttggacaagagacgtggccgggaccctgagatggggggaaagccgagaaggaagaaccctcaggaaggcctgtacaatgaactgcagaaagataagatggcggaggcctacagtgagattgggatgaaaggcgagcgccggaggggcaaggggcacgatggcctttaccagggtctcagtacagccaccaaggacacctacgacgcccttcacatgcaggccctgccccctcgctaa

SEQ ID NO: 8 - DNA, 2427 bp, Artificial Sequence
atggtgagcaagggcgaggagctgttcaccggggtggtgcccatcctggtcgagctggacggcgacgtaaacggccacaagttcagcgtgtccggcgagggcgagggcgatgccacctacggcaagctgaccctgaagttcatctgcaccaccggcaagctgcccgtgccctggcccaccctcgtgaccaccctgacctacggcgtgcagtgcttcagccgctaccccgaccacatgaagcagcacgacttcttcaagtccgccatgcccgaaggctacgtccaggagcgcaccatcttcttcaaggacgacggcaactacaagacccgcgccgaggtgaagttcgagggcgacaccctggtgaaccgcatcgagctgaagggcatcgacttcaaggaggacggcaacatcctggggcacaagctggagtacaactacaacagccacaacgtctatatcatggccgacaagcagaagaacggcatcaaggtgaacttcaagatccgccacaacatcgaggacggcagcgtgcagctcgccgaccactaccagcagaacacccccatcggcgacggccccgtgctgctgcccgacaaccactacctgagcacccagtccgccctgagcaaagaccccaacgagaagcgcgatcacatggtcctgctggagttcgtgaccgccgccgggatcactctcggcatggacgagctgtacaagggaagcggagagggcagaggaagtctgctaacatgcggtgacgtcgaggagaatcctggacctatgcttctcctggtgacaagccttctgctctgtgagttaccacacccagcattcctcctgatcccatacccctacgacgtgcccgactacgcccaggtacaactgcagcagtctgggcctgagctggagaagcctggcgcttcagtgaagatatcctgcaaggcttctggttactcattcactggctacaccatgaactgggtgaagcagagccatggaaagagccttgagtggattggacttattactccttacaatggtgcttctagctacaaccagaagttcaggggcaaggccacattaactgtagacaagtcatccagcacagcctacatggacctcctcagtctgacatctgaagactctgcagtctatttctgtgcaagggggggttacgacgggaggggttttgactactggggccaagggaccacggtcaccgtctcctcaggtggaggcggttcaggcggcggtggctctagcggtggtggatcggacatcgagctcactcagtctccagcaatcatgtctgcatctccaggggagaaggtcaccatgacctgcagtgccagctcaagtgtaagttacatgcactggtaccagcagaagtcaggcacctcccccaaaagatggatttatgacacatccaaactggcttctggagtcccaggtcgcttcagtggcagtgggtctggaaactcttactctctcacaatcagcagcgtggaggctgaagatgatgcaacttattactgccagcagtggagtaagcaccctctcacgtacggtgctgggacaaagttggaaatcaaagcggccgcaattgaagttatgtatcctcctccttacctagacaatgagaagagcaatggaaccattatccatgtgaaagggaaacacctttgtccaagtcccctatttcccggaccttctaagcccttttgggtgctggtggtggttgggggagtcctggcttgctatagcttgctagtaacagtggcctttattattttctgggtgaagaatagaaaggccaaggccaagcctgtgacacgaggagcgggtgctggcggcaggcaaaggggacaaaacaaggagaggccaccacctgttcccaacccagactatgagcccatccggaaaggccagcgggacctgtattctggcctgaatcagagacgcatcaggagtaagaggagcaggctcctgcacagtgactacatgaacatgactccccgccgccccgggcccacccgcaagcattaccagccctatgccccaccacgcgacttcgcagcctatcgctccagagtgaagttcagcaggagcgcagacgcccccgcgtaccagcagggccagaaccagctctataacgagctcaatctaggacgaagagaggagtacgatgttttggacaagagacgtggccgggaccctgagatggggggaaagccgagaaggaagaaccctcaggaaggcctgtacaatgaactgcagaaagataagatggcggaggcctacagtgagattgggatgaaaggcgagcgccggaggggcaaggggcacgatggcctttaccagggtctcagtacagccaccaaggacacctacgacgcccttcacatgcaggccctgccccctcgctaa

SEQ ID NO: 9 - DNA, 720 bp, Artificial Sequence
caggtacaactgcagcagtctgggcctgagctggagaagcctggcgcttcagtgaagatatcctgcaaggcttctggttactcattcactggctacaccatgaactgggtgaagcagagccatggaaagagccttgagtggattggacttattactccttacaatggtgcttctagctacaaccagaagttcaggggcaaggccacattaactgtagacaagtcatccagcacagcctacatggacctcctcagtctgacatctgaagactctgcagtctatttctgtgcaagggggggttacgacgggaggggttttgactactggggccaagggaccacggtcaccgtctcctcaggtggaggcggttcaggcggcggtggctctagcggtggtggatcggacatcgagctcactcagtctccagcaatcatgtctgcatctccaggggagaaggtcaccatgacctgcagtgccagctcaagtgtaagttacatgcactggtaccagcagaagtcaggcacctcccccaaaagatggatttatgacacatccaaactggcttctggagtcccaggtcgcttcagtggcagtgggtctggaaactcttactctctcacaatcagcagcgtggaggctgaagatgatgcaacttattactgccagcagtggagtaagcaccctctcacgtacggtgctgggacaaagttggaaatcaaa

SEQ ID NO: 10 - protein, 240 aa, Artificial Sequence
QVQLQQSGPELEKPGASVKISCKASGYSFTGYTMNWVKQSHGKSLEWIGLITPYNGASSYNQKFRGKATLTVDKSSSTAYMDLLSLTSEDSAVYFCARGGYDGRGFDYWGQGTTVTVSSGGGGSGGGGSSGGGSDIELTQSPAIMSASPGEKVTMTCSASSSVSYMHWYQQKSGTSPKRWIYDTSKLASGVPGRFSGSGSGNSYSLTISSVEAEDDATYYCQQWSKHPLTYGAGTKLEIK